European Patent Application EP 4 538 382 A1, published April 16, 2025. Title: Carotenoid production. Applicant: Faculty of Biology & CeBiTec Universitaet Bielefeld. Application EP. The sequence listing filed with the application follows.

SEQUENCE LISTING (18 sequences)

SEQ ID NO: 1 - protein, 841 aa, Pantoea ananatis
MQPHYDLILVGAGLANGLIALRLQQQQPDMRILLIDAAPQAGGNHTWSFHHDDLTESQHRWIAPLVVHHWPDYQVRFPTRRRKLNSGYFCITSQRFAEVLQRQFGPHLWMDTAVAEVNAESVRLKKGQVIGARAVIDGRGYAANSALSVGFQAFIGQEWRLSHPHGLSSPIIMDATVDQQNGYRFVYSLPLSPTRLLIEDTHYIDNATLDPECARQNICDYAAQQGWQLQTLLREEQGALPITLSGNADAFWQQRPLACSGLRAGLFHPTTGYSLPLAVAVADRLSALDVFTSASIHHAITHFARERWQQQGFFRMLNRMLFLAGPADSRWRVMQRFYGLPEDLIARFYAGKLTLTDRLRILSGKPPVPVLAALQAIMTTHRGSGSSGGPSGTIWTLYYVCLTLVTIGLMEVYAWWAHKFIMHGKFGWGWHKSHHEETEGWFEKNDLYAVVFAGFAIALFMVGHFLSPTLLAIAWGITLYGLLYFVAHDGLVHQRWPFNYVPHRGYAKRLVQAHRLHHAVEGREHCVSFGFLYAPPIEKLKRDLRESGILERERIERSLDQQGSAHAPVRGGGGSGGPGSTLSPTSRLIPASALPRSTPADSPKIRPYQTTIGLTLCAVLLASWFAIHVSAIFFLDINFSTLPLAPLITVFQCWLTVGLFILAHDAMHGSLAPGRTRLNAVIGGFILFVYAGFAWKKIRDAHFAHHDAPGTPADPDFYADDPENFWPWFGTFFSRYFGWRSVAFVSTVVTFYLVILDASVTNVVLFYGLPSLLSSLQLFYFGTYRPHRHEESGTFADAHNTRSSEFGYVASLFSCFHFGYHHEHHLAPWTPWWALPHTRQS

SEQ ID NO: 2 - protein, 262 aa, Fulvimarina pelagi
MTLSPTSRLIPASALPRSTPADSPKIRPYQTTIGLTLCAVLLASWFAIHVSAIFFLDINFSTLPLAPLITVFQCWLTVGLFILAHDAMHGSLAPGRTRLNAVIGGFILFVYAGFAWKKIRDAHFAHHDAPGTPADPDFYADDPENFWPWFGTFFSRYFGWRSVAFVSTVVTFYLVILDASVTNVVLFYGLPSLLSSLQLFYFGTYRPHRHEESGTFADAHNTRSSEFGYVASLFSCFHFGYHHEHHLAPWTPWWALPHTRQS

SEQ ID NO: 3 - protein, 179 aa, Fulvimarina pelagi
MTIWTLYYVCLTLVTIGLMEVYAWWAHKFIMHGKFGWGWHKSHHEETEGWFEKNDLYAVVFAGFAIALFMVGHFLSPTLLAIAWGITLYGLLYFVAHDGLVHQRWPFNYVPHRGYAKRLVQAHRLHHAVEGREHCVSFGFLYAPPIEKLKRDLRESGILERERIERSLDQQGSAHAPVR

SEQ ID NO: 4 - DNA, 1149 bp, Pantoea ananatis
  source 1..1149: mol_type = genomic DNA
atgcaaccgcattatgatctgattctcgtgggggctggactcgcgaatggccttatcgccctgcgtcttcagcagcagcaacctgatatgcgtattttgcttatcgacgccgcaccccaggcgggcgggaatcatacgtggtcatttcaccacgatgatttgactgagagccaacatcgttggatagctccgctggtggttcatcactggcccgactatcaggtacgctttcccacacgccgtcgtaagctgaacagcggctacttttgtattacttctcagcgtttcgctgaggttttacagcgacagtttggcccgcacttgtggatggataccgcggtcgcagaggttaatgcggaatctgttcggttgaaaaagggtcaggttatcggtgcccgcgcggtgattgacgggcggggttatgcggcaaattcagcactgagcgtgggcttccaggcgtttattggccaggaatggcgattgagccacccgcatggtttatcgtctcccattatcatggatgccacggtcgatcagcaaaatggttatcgcttcgtgtacagcctgccgctctcgccgaccagattgttaattgaagacacgcactatattgataatgcgacattagatcctgaatgcgcgcggcaaaatatttgcgactatgccgcgcaacagggttggcagcttcagacactgctgcgagaagaacagggcgccttacccattactctgtcgggcaatgccgacgcattctggcagcagcgccccctggcctgtagtggattacgtgccggtctgttccatcctaccaccggctattcactgccgctggcggttgccgtggccgaccgcctgagtgcacttgatgtctttacgtcggcctcaattcaccatgccattacgcattttgcccgcgagcgctggcagcagcagggctttttccgcatgctgaatcgcatgctgtttttagccggacccgccgattcacgctggcgggttatgcagcgtttttatggtttacctgaagatttaattgcccgtttttatgcgggaaaactcacgctgaccgatcggctacgtattctgagcggcaagccgcctgttccggtattagcagcattgcaagccattatgacgactcatcgttaa

SEQ ID NO: 5 - DNA, 789 bp, Fulvimarina pelagi
  source 1..789: mol_type = genomic DNA
atgaccctcagcccaacctcacgcctgatcccggcaagtgcgttaccgcgatccacacccgccgactcacccaaaatcagaccctaccaaacgacgattggcctgacgctctgtgccgtgctgctggcatcgtggttcgcaatacacgtctcagcgatattcttcctcgacatcaatttcagcacgttgcctctcgcaccattgatcacggtgttccagtgctggttgacggtggggcttttcatcctggctcacgacgccatgcatggttcgctggcgccgggtcgaacgcgtttgaatgccgtaatcggcgggttcatcctgttcgtctacgcgggatttgcgtggaaaaagatcagagatgctcacttcgcacaccacgacgcacccggtacaccggccgacccggatttctacgcagatgatccggagaatttctggccttggttcggcaccttcttctcacgttatttcggatggagatcggtcgcattcgtctcgaccgtcgtgacgttttatctcgtcatactggatgcatctgtgacgaacgtggttctattttacggcttgccgtcactgctttcgtcattgcagctcttctacttcggaacctaccgcccgcatcgacacgaagaatcgggcacctttgccgacgcgcataacacacgttcgagcgaattcggttacgtggcctcgctattctcctgcttccattttggctaccaccatgagcaccatttggcgccatggacgccttggtgggctctgccgcatactcgccagtcctaa

SEQ ID NO: 6 - DNA, 540 bp, Fulvimarina pelagi
  source 1..540: mol_type = genomic DNA
atgacgatctggactctctactacgtctgtctcaccctcgtcacgatcggtttgatggaggtttatgcatggtgggcgcacaagttcatcatgcatggcaaattcggttggggctggcataagtcccaccacgaggaaaccgaagggtggttcgagaagaacgatctctacgctgtcgttttcgccggcttcgcgatagcgctgttcatggtcggacatttcctttctccgaccctgctcgccatcgcctggggcatcacgctttacggattactctacttcgttgcccatgatggacttgtccatcagcgctggccgttcaactacgtgccgcatcgaggttatgcaaaacgcctggttcaagctcatcgtctgcaccatgcggtggaaggccgcgagcactgcgtctcgttcggctttctctatgcgccgccgattgaaaagctgaagcgcgatttgcgtgagtccggaattctcgaacgggagcgcatcgagcggtctctggaccagcaaggctccgcccacgcgccggttcggtaa

SEQ ID NO: 7-13 - skipped (7 entries)

SEQ ID NO: 14 - DNA, 588 bp, Corynebacterium glutamicum
  source 1..588: mol_type = genomic DNA
atgctgaatatgcaggaaccagataaaatccatccggcagaacctacacttcgtaatatttatgacgttaaaactagtgatcccaaaagtgaattagttgatcgttctggcatgtcggaagaagacattgcgcaaattgggcggctaatgaaatcgttggccagtcttcgcgatgtggaacgtagtattggtgaagcctcggcacgttatatggagctaagtgcccctgatatgcgagctttgcactatttgattgtggcgggcaatgcgggcgaagtggtgactccaggaatgcttggagctcaccttaagctttccccggcatctgtaacaaagacgcttaataggctagaaaaaggtgggcatattgttcgtaatgtgcaccccgtcgaccgcagggctttcgccctcatggtcactgatgccactcgtggagaggcgatgcggacgcttggtaagcatcaggcgcgtcgttttgatgctgctaaacgattaactccacaagagcgtgaagtggttatccgattccttcaggatatggcacaggagttatcccttaataatgcaccatggctcaacacggagtag

SEQ ID NO: 15 - protein, 195 aa, Corynebacterium glutamicum
MLNMQEPDKIHPAEPTLRNIYDVKTSDPKSELVDRSGMSEEDIAQIGRLMKSLASLRDVERSIGEASARYMELSAPDMRALHYLIVAGNAGEVVTPGMLGAHLKLSPASVTKTLNRLEKGGHIVRNVHPVDRRAFALMVTDATRGEAMRTLGKHQARRFDAAKRLTPQEREVVIRFLQDMAQELSLNNAPWLNTE

SEQ ID NO: 16 - DNA, 1523 bp, Corynebacterium glutamicum
  source 1..1523: mol_type = genomic DNA
tgtggagagtttgatcctggctcaggacgaacgctggcggcgtgcttaacacatgcaagtcgaacgctgaaaccggagcttgctttggtggatgagtggcgaacgggtgagtaacacgtgggtgatctgccctacactttgggataagcctgggaaactgggtctaataccgaatattcacaccaccgtaggggtggtgtggaaagctttatgcggtgtgggatgagcctgcggcctatcagcttgttggtggggtaatggcctaccaaggcgtcgacgggtagccggcctgagagggtgtacggccacattgggactgagacacggcccagactcctacgggaggcagcagtggggaatattgcacaatgggcgcaagcctgatgcagcgacgccgcgtgggggatgaaggccttcgggttgtaaactcctttcgctagggacgaagccttatggtgacggtacctggagaagaagcaccggctaactacgtgccagcagccgcggtaatacgtagggtgcgagcgttgtccggaattactgggcgtaaagagctcgtaggtggtttgtcgcgtcgtctgtgaaatcccggggcttaacttcgggcgtgcaggcgatacgggcataacttgagtgctgtaggggagactggaattcctggtgtagcggtgaaatgcgcagatatcaggaggaacaccaatggcgaaggcaggtctctgggcagtaactgacgctgaggagcgaaagcatgggtagcgaacaggattagataccctggtagtccatgccgtaaacggtgggcgctaggtgtaggggtcttccacgacttctgtgccgcagctaacgcattaagcgccccgcctggggagtacggccgcaaggctaaaactcaaaggaattgacgggggcccgcacaagcggcggagcatgtggattaattcgatgcaacgcgaagaaccttacctgggcttgacatggaccggatcggcgtagagatacgttttcccttgtggtcggttcacaggtggtgcatggttgtcgtcagctcgtgtcgtgagatgttgggttaagtcccgcaacgagcgcaacccttgtcttatgttgccagcacattatggtgggtactcatgagagactgccggggttaactcggaggaaggtggggatgacgtcaaatcatcatgccccttatgtccagggcttcacacatgctacaatggtcggtacagcgagttgccacaccgtgaggtggagctaatctcttaaagccggcctcagttcggattggggtctgcaactcgaccccatgaagtcggagtcgctagtaatcgcagatcagcaacgctgcggtgaatacgttcccgggccttgtacacaccgcccgtcacgtcatgaaagttggtaacacccgaagccagtggcccaaccttttaggggggagctgtcgaaggtgggatcggcgattgggacgaagtcgtaacaaggtagccgtaccggaaggtgcggctggatcacctcctttc

SEQ ID NO: 17 - RNA, 1523 nt, Corynebacterium glutamicum
  source 1..1523: mol_type = rRNA
tgtggagagtttgatcctggctcaggacgaacgctggcggcgtgcttaacacatgcaagtcgaacgctgaaaccggagcttgctttggtggatgagtggcgaacgggtgagtaacacgtgggtgatctgccctacactttgggataagcctgggaaactgggtctaataccgaatattcacaccaccgtaggggtggtgtggaaagctttatgcggtgtgggatgagcctgcggcctatcagcttgttggtggggtaatggcctaccaaggcgtcgacgggtagccggcctgagagggtgtacggccacattgggactgagacacggcccagactcctacgggaggcagcagtggggaatattgcacaatgggcgcaagcctgatgcagcgacgccgcgtgggggatgaaggccttcgggttgtaaactcctttcgctagggacgaagccttatggtgacggtacctggagaagaagcaccggctaactacgtgccagcagccgcggtaatacgtagggtgcgagcgttgtccggaattactgggcgtaaagagctcgtaggtggtttgtcgcgtcgtctgtgaaatcccggggcttaacttcgggcgtgcaggcgatacgggcataacttgagtgctgtaggggagactggaattcctggtgtagcggtgaaatgcgcagatatcaggaggaacaccaatggcgaaggcaggtctctgggcagtaactgacgctgaggagcgaaagcatgggtagcgaacaggattagataccctggtagtccatgccgtaaacggtgggcgctaggtgtaggggtcttccacgacttctgtgccgcagctaacgcattaagcgccccgcctggggagtacggccgcaaggctaaaactcaaaggaattgacgggggcccgcacaagcggcggagcatgtggattaattcgatgcaacgcgaagaaccttacctgggcttgacatggaccggatcggcgtagagatacgttttcccttgtggtcggttcacaggtggtgcatggttgtcgtcagctcgtgtcgtgagatgttgggttaagtcccgcaacgagcgcaacccttgtcttatgttgccagcacattatggtgggtactcatgagagactgccggggttaactcggaggaaggtggggatgacgtcaaatcatcatgccccttatgtccagggcttcacacatgctacaatggtcggtacagcgagttgccacaccgtgaggtggagctaatctcttaaagccggcctcagttcggattggggtctgcaactcgaccccatgaagtcggagtcgctagtaatcgcagatcagcaacgctgcggtgaatacgttcccgggccttgtacacaccgcccgtcacgtcatgaaagttggtaacacccgaagccagtggcccaaccttttaggggggagctgtcgaaggtgggatcggcgattgggacgaagtcgtaacaaggtagccgtaccggaaggtgcggctggatcacctcctttc

SEQ ID NO: 18 - DNA, 200 bp, Corynebacterium glutamicum
  source 1..200: mol_type = other DNA
tggccgttaccctgcgaatgtccacagggtagctggtagtttgaaaatcaacgccgttgcccttaggattcagtaactggcacattttgtaatgcgctagatctgtgtgctcagtcttccaggctgcttatcacagtgaaagcaaaaccaattcgtggctgcgaaagtcgtagccaccacgaagtccaggaggacataca